European Patent Application EP 4 190 810 A1, published June 7, 2023. Title: Neutralizing antibodies against SARS-related coronavirus. Applicant: Universität zu Köln. The sequence listing filed with the application follows.

SEQUENCE LISTING (152 sequences)

SEQ ID NO: 1 - protein, 123 aa, Artificial Sequence
  Heavy chain V domain of R200-1B9
QMQLVQSGPEVKKPGTSVKVSCKASGFTFDSSAVQWVRQARGQRLEWIGWIVVGSGNTNYAQKFQERVTITRDVSTNTAYMELRSLGSEDTAVYFCAAPHCNRTTCYDAFDLWGQGTMVTVSS

SEQ ID NO: 2 - protein, 108 aa, Artificial Sequence
  Light chain V domain of R200-1B9
EIVLTQSPGTLSLSPGERATLSCRASQSVRSSYLAWYQQKPGQAPRLLIYGPSSRATGIPDRFSGSGSGTDFTLTINRLEPEDFAVYYCQQYDRSPWTFGQGTKVEIK

SEQ ID NO: 3 - protein, 117 aa, Artificial Sequence
  Heavy chain V domain of R207-2F11
EVQLVESGGGLIQPGGSLRLSCAASGLIVSSNYMNWVRQAPGMGLEWVSVIYPGGTTYYADSVKGRFTISRDNSKNTLFLQMNSLRIDDTALYYCARDLVYRGMDVWGQGTTVTVSS

SEQ ID NO: 4 - protein, 107 aa, Artificial Sequence
  Light chain V domain of R207-2F11
KIQMTQSPSSLSASVGDRVIITCQASQDINKYLHWYQQKPGEAPKLVIYDASNLETGVPSRFSGSGSGTDFTFTISSLQPEDLARYYCQQYDNLPPTFGGGTKVEIK

SEQ ID NO: 5 - protein, 117 aa, Artificial Sequence
  Heavy chain V domain of R40-1G8
EVQLVESGGGLVQPGGSLRLSCAASGLTVSSNYMRWVRQAPGKGLEWVSLIYAGGSTFYADSVKGRFIISRHNSKNILYLQMNSLRAEDTAVYFCARDLYVFGMDVWGQGTAVTVSA

SEQ ID NO: 6 - protein, 107 aa, Artificial Sequence
  Light chain V domain of R40-1G8
DIQLTQSPSFLSASVGDRVTITCRASQGISSYLAWYQQKPGRAPKLLIYAASTLQSGVPSRFSGSGSGTVFTLTISSLQPEDFATYYCQQLNSDSSTFGQGTKLEIK

SEQ ID NO: 7 - protein, 117 aa, Artificial Sequence
  Heavy chain V domain of R568-2G5
EVQLVESGGGLIQPGGSLRLSCAASGVTVSSNYMTWVRQAPGKGLEWVSVIYSGGSTFYADSVKGRFTISRDDSMNTLYLQMSNVRAEDTAVYYCARDLYYYGMDVWGQGTTVTVSS

SEQ ID NO: 8 - protein, 109 aa, Artificial Sequence
  Light chain V domain of R568-2G5
DIQLTQSPSFLSASVGDRVTITCRASQGIGNYLAWYQQKPGKAPKLLIYAASTLQSGVPSRFSGSGSGTEFTLTISSLQPEDLATYYCQQVNSYPPECTFGQGTKLEIK

SEQ ID NO: 9 - protein, 117 aa, Artificial Sequence
  Heavy chain V domain of R568-2B11
EVQLVESGGGLIQPGGSLRLSCAASGLIVSSNYMSWVRQAPGKGLEWVSIIYAGGSTFYADSVKGRFTISRDNSKNTLYLQMNSLRAEDTAVYYCTRDLVYYGMDVWGQGTTVTVSS

SEQ ID NO: 10 - protein, 108 aa, Artificial Sequence
  Light chain V domain of R568-2B11
DIQLTQSPSFLSASVGDRITLTCRASQGISNYLAWYQQKPGKAPKLLIYAASTLQGGVPSRFSGSGSGTEFTLTISSLQPEDFATYYCQQLNSYPPDTFGQGTKLEIK

SEQ ID NO: 11 - protein, 117 aa, Artificial Sequence
  Heavy chain V domain of R207-2G4
EVQLVESGGGLIQPGGSLRLSCAASGLIVSSNYMNWVRQAPGKGLEWVSVLYSGGSTFYADSVKGRFTISRDNSKNTLHLQMNSLRVEDTAVYYCARDLVAYGMDVWGQGTTVTVSS

SEQ ID NO: 12 - protein, 103 aa, Artificial Sequence
  Light chain V domain of R207-2G4
DIQLTQSPSFLSASVGDRVTITCRASQGISSHLAWYQQKPGKAPKLLIFAASTLQSGVPSRFSGSGSGTEFSLTISSLQPADFATYFCQHLEMFGQGTKVEIK

SEQ ID NO: 13 - protein, 117 aa, Artificial Sequence
  Heavy chain V domain of R40-1C8
EVQLVESGGGLVQPGGSLRLSCAASGVTVSRNYMSWVRQAPGKGLEWVSVIYAGGSTFYADSVKGRFTISRHNSKNTLYLQMNSLRVEDTAVYYCVRDLVDYGMDVWGQGTTVTVSS

SEQ ID NO: 14 - protein, 108 aa, Artificial Sequence
  Light chain V domain of R40-1C8
DIQLTQSPSFLSASVGDRVTITCRASQGINSYLAWYQQKPGKAPKLLIYGASTLQSGVPSRFSGSGSGTEFTLTISSLQPEDFATYYCQQLNSYSRDTFGQGTKLEIK

SEQ ID NO: 15 - protein, 117 aa, Artificial Sequence
  Heavy chain V domain of R568-2B9
EVQLVESGGGLAQPGGSLRLSCAASGITVSSNYMSWVRQAPGKGLEWVSVMYAGGSTFYSDSVKGRFTISRDGPKNTLYLHMHSLRAEDTAVYYCARDLVHYGMDVWGQGTTVTVSS

SEQ ID NO: 16 - protein, 108 aa, Artificial Sequence
  Light chain V domain of R568-2B9
DIQLTQSPAFLSASVGDRVRITCRASQGISSYLAWYQQKPGKAPKLLIYAASTLQSGVPSRFSGSGSGTEFTLTISSLQPEDFATYYCQQLTNYPPDTFGQGTKLEIK

SEQ ID NO: 17 - protein, 117 aa, Artificial Sequence
  Heavy chain V domain of R568-1B3
EVQLVESGGGLIQPGGSLRLSCAASGLIVSSNYMTWVRQAPGKGLEWVSVLYAGGSSFYADSVKGRFTISRDNSKNTLFLQMNSLRAEDTAVYYCARDLVAYGMDVWGQGTTVSVSS

SEQ ID NO: 18 - protein, 107 aa, Artificial Sequence
  Light chain V domain of R568-1B3
DIQLTQSPSFLSASVGGRVTITCRASQGISSSLAWYQQKPGKAPKLLIYGASTLRTGVPSRFSGSGSGTEFTLTISSLQPEDFATYYCQQLNSDLYTFGQGTKLEIK

SEQ ID NO: 19 - protein, 117 aa, Artificial Sequence
  Heavy chain V domain of R568-2E1
EVQLVESGGGLIQPGGSLRLSCAASGLTVSSNYMNWVRQAPGKGLEWVSVIYSGGTTYYADSVKGRFTISRDNSKNTLYLQMNNLRDEDTAMYYCARDLIVYGMDVWGQGTPVTVSS

SEQ ID NO: 20 - protein, 107 aa, Artificial Sequence
  Light chain V domain of R568-2E1
DIQLTQSPSFLSASVGDRVTITCRASQGISNYLAWYQQKPGKAPKLLIYGASTLQSGVPSRFSGSGSGTEFTLTISSLQPEDFATYYCQQLNSDFFTFGPGTKVDIK

SEQ ID NO: 21 - protein, 118 aa, Artificial Sequence
  Heavy chain V domain or R568-1G9
EVQLVESGGGLVQPGGSLRLSCAASGITVSSNYMSWVRQAPGKGLEWVSVIYSGGSTFYTDSVKGRFTISRDNSKNTLYLQMNSLRAEDTAVYYCARDLVVLYGMDVWGQGTTVTVSS

SEQ ID NO: 22 - protein, 110 aa, Artificial Sequence
  Light chain V domain of R568-1G9
QSVLTQPPSVSGAPGQRVTISCTGNSSNIGAGYDVHWYQQLPGTAPKLLIYGNSNRPSGVPDRFSGSKSGTSASLAITGLQAEDEADYYCQSYDSSLSALFGTGTKVTVL

SEQ ID NO: 23 - protein, 121 aa, Artificial Sequence
  Heavy chain V domain of R121-1F1
QVQLVESGGGVVQPERSLRLSCAASGFTFSRDGMHWVRRAPGKGLEWVAVISYDGSNKVYAESVKGRFTVSRDSSKNTVYLQMNSLRAEDTAVYYCAKDGPQAFGTYFDYWGQGTLVIVSS

SEQ ID NO: 24 - protein, 111 aa, Artificial Sequence
  Light chain V domain of R121-1F1
QSALTQPPSVSGAPGQRVTISCTGSSSNIGSGYVVHWYQHLPNTAPKLLIFGNNNRPSGVPDRFSGSKSGTSASLAITGLQAEDEADYYCQSYDSRLSGVVFGGGTKLTVL

SEQ ID NO: 25 - protein, 123 aa, Artificial Sequence
  Heavy chain V domain of R259-1B9
QMHLVQSGPEVKKPGTSVKVSCKASGFTFSSSAVQWVRQARGQHLEWIGWIVVGSGNTNYGQKFQERVTITRDLSTSTVYMELISLRSEDTAVYFCAAPYCTGGSCFDAFDIWGQGTMVTVSS

SEQ ID NO: 26 - protein, 108 aa, Artificial Sequence
  Light chain V domain of R259-1B9
ETVLTQSPGTLSLSPGERATLSCRASQSVRSSYLAWYQQKPGQAPRLVIYGPSTRATGIPDRFSGSGSGTDFTLTISRLEPEDFAVYYCQQYGSSPWTFGQGTKVEIK

SEQ ID NO: 27 - protein, 8 aa, Artificial Sequence
  CDR-H1 of R200-1B9
GFTFDSSA

SEQ ID NO: 28 - protein, 8 aa, Artificial Sequence
  CDR-H2 of R200-1B9
IVVGSGNT

SEQ ID NO: 29 - protein, 16 aa, Artificial Sequence
  CDR-H3 of R200-1B9
AAPHCNRTTCYDAFDL

SEQ ID NO: 30 - protein, 7 aa, Artificial Sequence
  CDR-L1 of R200-1B9
QSVRSSY

SEQ ID NO: 31 - protein, 3 aa, Artificial Sequence
  CDR-L2 of R200-1B9
GPS

SEQ ID NO: 32 - protein, 9 aa, Artificial Sequence
  CDR-L3 of R200-1B9
QQYDRSPWT

SEQ ID NO: 33 - protein, 8 aa, Artificial Sequence
  CDR-H1 of R207-2F11
GLIVSSNY

SEQ ID NO: 34 - protein, 7 aa, Artificial Sequence
  CDR-H2 of R207-2F11
IYPGGTT

SEQ ID NO: 35 - protein, 11 aa, Artificial Sequence
  CDR-H3 of R207-2F11
ARDLVYRGMDV

SEQ ID NO: 36 - protein, 6 aa, Artificial Sequence
  CDR-L1 of R207-2F11
QDINKY

SEQ ID NO: 37 - protein, 3 aa, Artificial Sequence
  CDR-L2 of R207-2F11
DAS

SEQ ID NO: 38 - protein, 9 aa, Artificial Sequence
  CDR-L3 of R207-2F11
QQYDNLPPT

SEQ ID NO: 39 - protein, 8 aa, Artificial Sequence
  CDR-H1 of R40-1G8
GLTVSSNY

SEQ ID NO: 40 - protein, 7 aa, Artificial Sequence
  CDR-H2 of R40-1G8
IYAGGST

SEQ ID NO: 41 - protein, 11 aa, Artificial Sequence
  CDR-H3 of R40-1G8
ARDLYVFGMDV

SEQ ID NO: 42 - protein, 6 aa, Artificial Sequence
  CDR-L1 of R40-1G8
QGISSY

SEQ ID NO: 43 - protein, 3 aa, Artificial Sequence
  CDR-L2 of R40-1G8
AAS

SEQ ID NO: 44 - protein, 9 aa, Artificial Sequence
  CDR-L3 of R40-1G8
QQLNSDSST

SEQ ID NO: 45 - protein, 8 aa, Artificial Sequence
  CDR-H1 of R568-2G5
GVTVSSNY

SEQ ID NO: 46 - protein, 7 aa, Artificial Sequence
  CDR-H2 of R568-2G5
IYSGGST

SEQ ID NO: 47 - protein, 11 aa, Artificial Sequence
  CDR-H3 of R568-2G5
ARDLYYYGMDV

SEQ ID NO: 48 - protein, 6 aa, Artificial Sequence
  CDR-L1 of R568-2G5
QGIGNY

SEQ ID NO: 49 - protein, 3 aa, Artificial Sequence
  CDR-L2 of R568-2G5
AAS

SEQ ID NO: 50 - protein, 11 aa, Artificial Sequence
  CDR-L3 of R568-2G5
QQVNSYPPECT

SEQ ID NO: 51 - protein, 8 aa, Artificial Sequence
  CDR-H1 of R568-2B11
GLIVSSNY

SEQ ID NO: 52 - protein, 7 aa, Artificial Sequence
  CDR-H2 of R568-2B11
IYAGGST

SEQ ID NO: 53 - protein, 11 aa, Artificial Sequence
  CDR-H3 of R568-2B11
TRDLVYYGMDV

SEQ ID NO: 54 - protein, 6 aa, Artificial Sequence
  CDR-L1 of R568-2B11
QGISNY

SEQ ID NO: 55 - protein, 3 aa, Artificial Sequence
  CDR-L2 of R568-2B11
AAS

SEQ ID NO: 56 - protein, 10 aa, Artificial Sequence
  CDR-L3 of R568-2B11
QQLNSYPPDT

SEQ ID NO: 57 - protein, 8 aa, Artificial Sequence
  CDR-H1 of R207-2G4
GLIVSSNY

SEQ ID NO: 58 - protein, 7 aa, Artificial Sequence
  CDR-H2 of R207-2G4
LYSGGST

SEQ ID NO: 59 - protein, 11 aa, Artificial Sequence
  CDR-H3 of R207-2G4
ARDLVAYGMDV

SEQ ID NO: 60 - protein, 6 aa, Artificial Sequence
  CDR-L1 of R207-2G4
QGISSH

SEQ ID NO: 61 - protein, 3 aa, Artificial Sequence
  CDR-L2 of R207-2G4
AAS

SEQ ID NO: 62 - protein, 5 aa, Artificial Sequence
  CDR-L3 of R207-2G4
QHLEM

SEQ ID NO: 63 - protein, 8 aa, Artificial Sequence
  CDR-H1 of R40-1C8
GVTVSRNY

SEQ ID NO: 64 - protein, 7 aa, Artificial Sequence
  CDR-H2 of R40-1C8
IYAGGST

SEQ ID NO: 65 - protein, 11 aa, Artificial Sequence
  CDR-H3 of R40-1C8
VRDLVDYGMDV

SEQ ID NO: 66 - protein, 6 aa, Artificial Sequence
  CDR-L1 of R40-1C8
QGINSY

SEQ ID NO: 67 - protein, 3 aa, Artificial Sequence
  CDR-L2 of R40-1C8
GAS

SEQ ID NO: 68 - protein, 10 aa, Artificial Sequence
  CDR-L3 of R40-1C8
QQLNSYSRDT

SEQ ID NO: 69 - protein, 8 aa, Artificial Sequence
  CDR-H1 of R568-2B9
GITVSSNY

SEQ ID NO: 70 - protein, 7 aa, Artificial Sequence
  CDR-H2 of R568-2B9
MYAGGST

SEQ ID NO: 71 - protein, 11 aa, Artificial Sequence
  CDR-H3 of R568-2B9
ARDLVHYGMDV

SEQ ID NO: 72 - protein, 6 aa, Artificial Sequence
  CDR-L1 of R568-2B9
QGISSY

SEQ ID NO: 73 - protein, 3 aa, Artificial Sequence
  CDR-L2 of R568-2B9
AAS

SEQ ID NO: 74 - protein, 10 aa, Artificial Sequence
  CDR-L3 of R568-2B9
QQLTNYPPDT

SEQ ID NO: 75 - protein, 8 aa, Artificial Sequence
  CDR-H1 of R568-1B3
GLIVSSNY

SEQ ID NO: 76 - protein, 7 aa, Artificial Sequence
  CDR-H2 of R568-1B3
LYAGGSS

SEQ ID NO: 77 - protein, 11 aa, Artificial Sequence
  CDR-H3 of R568-1B3
ARDLVAYGMDV

SEQ ID NO: 78 - protein, 6 aa, Artificial Sequence
  CDR-L1 of R568-1B3
QGISSS

SEQ ID NO: 79 - protein, 3 aa, Artificial Sequence
  CDR-L2 of R568-1B3
GAS

SEQ ID NO: 80 - protein, 9 aa, Artificial Sequence
  CDR-L3 of R568-1B3
QQLNSDLYT

SEQ ID NO: 81 - protein, 8 aa, Artificial Sequence
  CDR-H1 of R568-2E1
GLTVSSNY

SEQ ID NO: 82 - protein, 7 aa, Artificial Sequence
  CDR-H2 of R568-2E1
IYSGGTT

SEQ ID NO: 83 - protein, 11 aa, Artificial Sequence
  CDR-H3 of R568-2E1
ARDLIVYGMDV

SEQ ID NO: 84 - protein, 6 aa, Artificial Sequence
  CDR-L1 of R568-2E1
QGISNY

SEQ ID NO: 85 - protein, 3 aa, Artificial Sequence
  CDR-L2 of R568-2E1
GAS

SEQ ID NO: 86 - protein, 9 aa, Artificial Sequence
  CDR-L3 of R568-2E1
QQLNSDFFT

SEQ ID NO: 87 - protein, 8 aa, Artificial Sequence
  CDR-H1 of R568-1G9
GITVSSNY

SEQ ID NO: 88 - protein, 7 aa, Artificial Sequence
  CDR-H2 of R568-1G9
IYSGGST

SEQ ID NO: 89 - protein, 12 aa, Artificial Sequence
  CDR-H3 of R568-1G9
ARDLVVLYGMDV

SEQ ID NO: 90 - protein, 9 aa, Artificial Sequence
  CDR-L1 of R568-1G9
SSNIGAGYD

SEQ ID NO: 91 - protein, 3 aa, Artificial Sequence
  CDR-L2 of R568-1G9
GNS

SEQ ID NO: 92 - protein, 10 aa, Artificial Sequence
  CDR-L3 of R568-1G9
QSYDSSLSAL

SEQ ID NO: 93 - protein, 8 aa, Artificial Sequence
  CDR-H1 of R121-1F1
GFTFSRDG

SEQ ID NO: 94 - protein, 8 aa, Artificial Sequence
  CDR-H2 of R121-1F1
ISYDGSNK

SEQ ID NO: 95 - protein, 14 aa, Artificial Sequence
  CDR-H3 of R121-1F1
AKDGPQAFGTYFDY

SEQ ID NO: 96 - protein, 9 aa, Artificial Sequence
  CDR-L1 of R121-1F1
SSNIGSGYV

SEQ ID NO: 97 - protein, 3 aa, Artificial Sequence
  CDR-L2 of R121-1F1
GNN

SEQ ID NO: 98 - protein, 11 aa, Artificial Sequence
  CDR-L3 of R121-1F1
QSYDSRLSGVV

SEQ ID NO: 99 - protein, 8 aa, Artificial Sequence
  CDR-H1 of R259-1B9
GFTFSSSA

SEQ ID NO: 100 - protein, 8 aa, Artificial Sequence
  CDR-H2 of R259-1B9
IVVGSGNT

SEQ ID NO: 101 - protein, 16 aa, Artificial Sequence
  CDR-H3 of R259-1B9
AAPYCTGGSCFDAFDI

SEQ ID NO: 102 - protein, 7 aa, Artificial Sequence
  CDR-L1 of R259-1B9
QSVRSSY

SEQ ID NO: 103 - protein, 3 aa, Artificial Sequence
  CDR-L2 of R259-1B9
GPS

SEQ ID NO: 104 - protein, 9 aa, Artificial Sequence
  CDR-L3 of R259-1B9
QQYGSSPWT

SEQ ID NO: 105 - protein, 129 aa, Artificial Sequence
  Heavy chain V domain of R121-3G2
QLQLQESGPGLVKPSETLSLTCTVSGGSIASTYYYWGWIRQSPGKGLEWIANIHYNGSTYNKPSLKNRVTLSVDTSKNQFSLKLSSVTAADTAVYYCARYGPYYYDRSGSLLSDPFDNWGQGTLVTVSS

SEQ ID NO: 106 - protein, 108 aa, Artificial Sequence
  Light chain V domain of R121-3G2
EVVLTQSPGTLSLSPGERATLSCRASQGLSSSSLAWYQQRPGQAPRLLIYGASNRATGISDRFSGSGSGTDFTLSVSRLEPEDFAVYYCQQYSNSPLTFGQGTKVEIK

SEQ ID NO: 107 - protein, 131 aa, Artificial Sequence
  Heavy chain V domain of R40-1E1
QVQLVESGGGVVQPGRSLRLSCAASGFTFSRYGMNWVRQAPGKGLEWVAVIWYDGNNKYYADSVKGRFTISRDNSKTTLYLQMKSLRAEDTAVYYCARALQYYDILTGDYSVVRSDAFDIWGQGTMVTVSS

SEQ ID NO: 108 - protein, 108 aa, Artificial Sequence
  Light chain V domain of R40-1E1
EIVLTQSPGTLSLSPGERATLSCRASQSVSGTYLAWYQQKPGQAPRLLIYGASSRASGIPDRFSGSGSGTDFTLTISRLEPEDFAVYYCQQYGSSPLTFGGGTKVEIK

SEQ ID NO: 109 - protein, 10 aa, Artificial Sequence
  CDR-H1 of R121-3G2
GGSIASTYYY

SEQ ID NO: 110 - protein, 7 aa, Artificial Sequence
  CDR-H2 of R121-3G2
IHYNGST

SEQ ID NO: 111 - protein, 21 aa, Artificial Sequence
  CDR-H3 of R121-3G2
ARYGPYYYDRSGSLLSDPFDN

SEQ ID NO: 112 - protein, 7 aa, Artificial Sequence
  CDR-L1 of R121-3G2
QGLSSSS

SEQ ID NO: 113 - protein, 3 aa, Artificial Sequence
  CDR-L2 of R121-3G2
GAS

SEQ ID NO: 114 - protein, 9 aa, Artificial Sequence
  CDR-L3 of R121-3G2
QQYSNSPLT

SEQ ID NO: 115 - protein, 8 aa, Artificial Sequence
  CDR-H1 of R40-1E1
GFTFSRYG

SEQ ID NO: 116 - protein, 8 aa, Artificial Sequence
  CDR-H2 of R40-1E1
IWYDGNNK

SEQ ID NO: 117 - protein, 24 aa, Artificial Sequence
  CDR-H3 of R40-1E1
ARALQYYDILTGDYSVVRSDAFDI

SEQ ID NO: 118 - protein, 7 aa, Artificial Sequence
  CDR-L1 of R40-1E1
QSVSGTY

SEQ ID NO: 119 - protein, 3 aa, Artificial Sequence
  CDR-L2 of R40-1E1
GAS

SEQ ID NO: 120 - protein, 9 aa, Artificial Sequence
  CDR-L3 of R40-1E1
QQYGSSPLT

SEQ ID NO: 121 - protein, 453 aa, Artificial Sequence
  Complete heavy chain of antibody R200-1B9 with IGHG1*01
QMQLVQSGPEVKKPGTSVKVSCKASGFTFDSSAVQWVRQARGQRLEWIGWIVVGSGNTNYAQKFQERVTITRDVSTNTAYMELRSLGSEDTAVYFCAAPHCNRTTCYDAFDLWGQGTMVTVSSASTKGPSVFPLAPSSKSTSGGTAALGCLVKDYFPEPVTVSWNSGALTSGVHTFPAVLQSSGLYSLSSVVTVPSSSLGTQTYICNVNHKPSNTKVDKKVEPKSCDKTHTCPPCPAPELLGGPSVFLFPPKPKDTLMISRTPEVTCVVVDVSHEDPEVKFNWYVDGVEVHNAKTKPREEQYNSTYRVVSVLTVLHQDWLNGKEYKCKVSNKALPAPIEKTISKAKGQPREPQVYTLPPSRDELTKNQVSLTCLVKGFYPSDIAVEWESNGQPENNYKTTPPVLDSDGSFFLYSKLTVDKSRWQQGNVFSCSVMHEALHNHYTQKSLSLSPGK

SEQ ID NO: 122 - protein, 215 aa, Artificial Sequence
  Complete light chain of antibody R200-1B9 with IGKC*01
EIVLTQSPGTLSLSPGERATLSCRASQSVRSSYLAWYQQKPGQAPRLLIYGPSSRATGIPDRFSGSGSGTDFTLTINRLEPEDFAVYYCQQYDRSPWTFGQGTKVEIKRTVAAPSVFIFPPSDEQLKSGTASVVCLLNNFYPREAKVQWKVDNALQSGNSQESVTEQDSKDSTYSLSSTLTLSKADYEKHKVYACEVTHQGLSSPVTKSFNRGEC

SEQ ID NO: 123 - protein, 447 aa, Artificial Sequence
  Complete heavy chain of antibody R207-2F11 with IGHG1*01
EVQLVESGGGLIQPGGSLRLSCAASGLIVSSNYMNWVRQAPGMGLEWVSVIYPGGTTYYADSVKGRFTISRDNSKNTLFLQMNSLRIDDTALYYCARDLVYRGMDVWGQGTTVTVSSASTKGPSVFPLAPSSKSTSGGTAALGCLVKDYFPEPVTVSWNSGALTSGVHTFPAVLQSSGLYSLSSVVTVPSSSLGTQTYICNVNHKPSNTKVDKKVEPKSCDKTHTCPPCPAPELLGGPSVFLFPPKPKDTLMISRTPEVTCVVVDVSHEDPEVKFNWYVDGVEVHNAKTKPREEQYNSTYRVVSVLTVLHQDWLNGKEYKCKVSNKALPAPIEKTISKAKGQPREPQVYTLPPSRDELTKNQVSLTCLVKGFYPSDIAVEWESNGQPENNYKTTPPVLDSDGSFFLYSKLTVDKSRWQQGNVFSCSVMHEALHNHYTQKSLSLSPGK

SEQ ID NO: 124 - protein, 214 aa, Artificial Sequence
  Complete light chain of antibody R207-2F11 with IGKC*01
KIQMTQSPSSLSASVGDRVIITCQASQDINKYLHWYQQKPGEAPKLVIYDASNLETGVPSRFSGSGSGTDFTFTISSLQPEDLARYYCQQYDNLPPTFGGGTKVEIKRTVAAPSVFIFPPSDEQLKSGTASVVCLLNNFYPREAKVQWKVDNALQSGNSQESVTEQDSKDSTYSLSSTLTLSKADYEKHKVYACEVTHQGLSSPVTKSFNRGEC

SEQ ID NO: 125 - protein, 447 aa, Artificial Sequence
  Complete heavy chain of antibody R40-1G8 with IGHG1*01
EVQLVESGGGLVQPGGSLRLSCAASGLTVSSNYMRWVRQAPGKGLEWVSLIYAGGSTFYADSVKGRFIISRHNSKNILYLQMNSLRAEDTAVYFCARDLYVFGMDVWGQGTAVTVSAASTKGPSVFPLAPSSKSTSGGTAALGCLVKDYFPEPVTVSWNSGALTSGVHTFPAVLQSSGLYSLSSVVTVPSSSLGTQTYICNVNHKPSNTKVDKKVEPKSCDKTHTCPPCPAPELLGGPSVFLFPPKPKDTLMISRTPEVTCVVVDVSHEDPEVKFNWYVDGVEVHNAKTKPREEQYNSTYRVVSVLTVLHQDWLNGKEYKCKVSNKALPAPIEKTISKAKGQPREPQVYTLPPSRDELTKNQVSLTCLVKGFYPSDIAVEWESNGQPENNYKTTPPVLDSDGSFFLYSKLTVDKSRWQQGNVFSCSVMHEALHNHYTQKSLSLSPGK

SEQ ID NO: 126 - protein, 214 aa, Artificial Sequence
  Complete light chain of antibody R40-1G8 with IGKC*01
DIQLTQSPSFLSASVGDRVTITCRASQGISSYLAWYQQKPGRAPKLLIYAASTLQSGVPSRFSGSGSGTVFTLTISSLQPEDFATYYCQQLNSDSSTFGQGTKLEIKRTVAAPSVFIFPPSDEQLKSGTASVVCLLNNFYPREAKVQWKVDNALQSGNSQESVTEQDSKDSTYSLSSTLTLSKADYEKHKVYACEVTHQGLSSPVTKSFNRGEC

SEQ ID NO: 127 - protein, 447 aa, Artificial Sequence
  Complete heavy chain of antibody R568-2G5 with IGHG1*01
EVQLVESGGGLIQPGGSLRLSCAASGVTVSSNYMTWVRQAPGKGLEWVSVIYSGGSTFYADSVKGRFTISRDDSMNTLYLQMSNVRAEDTAVYYCARDLYYYGMDVWGQGTTVTVSSASTKGPSVFPLAPSSKSTSGGTAALGCLVKDYFPEPVTVSWNSGALTSGVHTFPAVLQSSGLYSLSSVVTVPSSSLGTQTYICNVNHKPSNTKVDKKVEPKSCDKTHTCPPCPAPELLGGPSVFLFPPKPKDTLMISRTPEVTCVVVDVSHEDPEVKFNWYVDGVEVHNAKTKPREEQYNSTYRVVSVLTVLHQDWLNGKEYKCKVSNKALPAPIEKTISKAKGQPREPQVYTLPPSRDELTKNQVSLTCLVKGFYPSDIAVEWESNGQPENNYKTTPPVLDSDGSFFLYSKLTVDKSRWQQGNVFSCSVMHEALHNHYTQKSLSLSPGK

SEQ ID NO: 128 - protein, 216 aa, Artificial Sequence
  Complete light chain of antibody R568-2G5 with IGKC*01
DIQLTQSPSFLSASVGDRVTITCRASQGIGNYLAWYQQKPGKAPKLLIYAASTLQSGVPSRFSGSGSGTEFTLTISSLQPEDLATYYCQQVNSYPPECTFGQGTKLEIKRTVAAPSVFIFPPSDEQLKSGTASVVCLLNNFYPREAKVQWKVDNALQSGNSQESVTEQDSKDSTYSLSSTLTLSKADYEKHKVYACEVTHQGLSSPVTKSFNRGEC

SEQ ID NO: 129 - protein, 447 aa, Artificial Sequence
  Complete heavy chain of antibody R568-2B11 with IGHG1*01
EVQLVESGGGLIQPGGSLRLSCAASGLIVSSNYMSWVRQAPGKGLEWVSIIYAGGSTFYADSVKGRFTISRDNSKNTLYLQMNSLRAEDTAVYYCTRDLVYYGMDVWGQGTTVTVSSASTKGPSVFPLAPSSKSTSGGTAALGCLVKDYFPEPVTVSWNSGALTSGVHTFPAVLQSSGLYSLSSVVTVPSSSLGTQTYICNVNHKPSNTKVDKKVEPKSCDKTHTCPPCPAPELLGGPSVFLFPPKPKDTLMISRTPEVTCVVVDVSHEDPEVKFNWYVDGVEVHNAKTKPREEQYNSTYRVVSVLTVLHQDWLNGKEYKCKVSNKALPAPIEKTISKAKGQPREPQVYTLPPSRDELTKNQVSLTCLVKGFYPSDIAVEWESNGQPENNYKTTPPVLDSDGSFFLYSKLTVDKSRWQQGNVFSCSVMHEALHNHYTQKSLSLSPGK

SEQ ID NO: 130 - protein, 215 aa, Artificial Sequence
  Complete light chain of antibody R568-2B11 with IGKC*01
DIQLTQSPSFLSASVGDRITLTCRASQGISNYLAWYQQKPGKAPKLLIYAASTLQGGVPSRFSGSGSGTEFTLTISSLQPEDFATYYCQQLNSYPPDTFGQGTKLEIKRTVAAPSVFIFPPSDEQLKSGTASVVCLLNNFYPREAKVQWKVDNALQSGNSQESVTEQDSKDSTYSLSSTLTLSKADYEKHKVYACEVTHQGLSSPVTKSFNRGEC

SEQ ID NO: 131 - protein, 447 aa, Artificial Sequence
  Complete heavy chain of antibody R207-2G4 with IGHG1*01
EVQLVESGGGLIQPGGSLRLSCAASGLIVSSNYMNWVRQAPGKGLEWVSVLYSGGSTFYADSVKGRFTISRDNSKNTLHLQMNSLRVEDTAVYYCARDLVAYGMDVWGQGTTVTVSSASTKGPSVFPLAPSSKSTSGGTAALGCLVKDYFPEPVTVSWNSGALTSGVHTFPAVLQSSGLYSLSSVVTVPSSSLGTQTYICNVNHKPSNTKVDKKVEPKSCDKTHTCPPCPAPELLGGPSVFLFPPKPKDTLMISRTPEVTCVVVDVSHEDPEVKFNWYVDGVEVHNAKTKPREEQYNSTYRVVSVLTVLHQDWLNGKEYKCKVSNKALPAPIEKTISKAKGQPREPQVYTLPPSRDELTKNQVSLTCLVKGFYPSDIAVEWESNGQPENNYKTTPPVLDSDGSFFLYSKLTVDKSRWQQGNVFSCSVMHEALHNHYTQKSLSLSPGK

SEQ ID NO: 132 - protein, 210 aa, Artificial Sequence
  Complete light chain of antibody R207-2G4 with IGKC*01
DIQLTQSPSFLSASVGDRVTITCRASQGISSHLAWYQQKPGKAPKLLIFAASTLQSGVPSRFSGSGSGTEFSLTISSLQPADFATYFCQHLEMFGQGTKVEIKRTVAAPSVFIFPPSDEQLKSGTASVVCLLNNFYPREAKVQWKVDNALQSGNSQESVTEQDSKDSTYSLSSTLTLSKADYEKHKVYACEVTHQGLSSPVTKSFNRGEC

SEQ ID NO: 133 - protein, 447 aa, Artificial Sequence
  Complete heavy chain of antibody R40-1C8 with IGHG1*01
EVQLVESGGGLVQPGGSLRLSCAASGVTVSRNYMSWVRQAPGKGLEWVSVIYAGGSTFYADSVKGRFTISRHNSKNTLYLQMNSLRVEDTAVYYCVRDLVDYGMDVWGQGTTVTVSSASTKGPSVFPLAPSSKSTSGGTAALGCLVKDYFPEPVTVSWNSGALTSGVHTFPAVLQSSGLYSLSSVVTVPSSSLGTQTYICNVNHKPSNTKVDKKVEPKSCDKTHTCPPCPAPELLGGPSVFLFPPKPKDTLMISRTPEVTCVVVDVSHEDPEVKFNWYVDGVEVHNAKTKPREEQYNSTYRVVSVLTVLHQDWLNGKEYKCKVSNKALPAPIEKTISKAKGQPREPQVYTLPPSRDELTKNQVSLTCLVKGFYPSDIAVEWESNGQPENNYKTTPPVLDSDGSFFLYSKLTVDKSRWQQGNVFSCSVMHEALHNHYTQKSLSLSPGK

SEQ ID NO: 134 - protein, 215 aa, Artificial Sequence
  Complete light chain of antibody R40-1C8 with with IGKC*01
DIQLTQSPSFLSASVGDRVTITCRASQGINSYLAWYQQKPGKAPKLLIYGASTLQSGVPSRFSGSGSGTEFTLTISSLQPEDFATYYCQQLNSYSRDTFGQGTKLEIKRTVAAPSVFIFPPSDEQLKSGTASVVCLLNNFYPREAKVQWKVDNALQSGNSQESVTEQDSKDSTYSLSSTLTLSKADYEKHKVYACEVTHQGLSSPVTKSFNRGEC

SEQ ID NO: 135 - protein, 447 aa, Artificial Sequence
  Complete heavy chain of antibody R568-2B9 with IGHG1*01
EVQLVESGGGLAQPGGSLRLSCAASGITVSSNYMSWVRQAPGKGLEWVSVMYAGGSTFYSDSVKGRFTISRDGPKNTLYLHMHSLRAEDTAVYYCARDLVHYGMDVWGQGTTVTVSSASTKGPSVFPLAPSSKSTSGGTAALGCLVKDYFPEPVTVSWNSGALTSGVHTFPAVLQSSGLYSLSSVVTVPSSSLGTQTYICNVNHKPSNTKVDKKVEPKSCDKTHTCPPCPAPELLGGPSVFLFPPKPKDTLMISRTPEVTCVVVDVSHEDPEVKFNWYVDGVEVHNAKTKPREEQYNSTYRVVSVLTVLHQDWLNGKEYKCKVSNKALPAPIEKTISKAKGQPREPQVYTLPPSRDELTKNQVSLTCLVKGFYPSDIAVEWESNGQPENNYKTTPPVLDSDGSFFLYSKLTVDKSRWQQGNVFSCSVMHEALHNHYTQKSLSLSPGK

SEQ ID NO: 136 - protein, 215 aa, Artificial Sequence
  Complete light chain of antibody R568-2B9 with with IGKC*01
DIQLTQSPAFLSASVGDRVRITCRASQGISSYLAWYQQKPGKAPKLLIYAASTLQSGVPSRFSGSGSGTEFTLTISSLQPEDFATYYCQQLTNYPPDTFGQGTKLEIKRTVAAPSVFIFPPSDEQLKSGTASVVCLLNNFYPREAKVQWKVDNALQSGNSQESVTEQDSKDSTYSLSSTLTLSKADYEKHKVYACEVTHQGLSSPVTKSFNRGEC

SEQ ID NO: 137 - protein, 447 aa, Artificial Sequence
  Complete heavy chain of antibody R568-1B3 with IGHG1*01
EVQLVESGGGLIQPGGSLRLSCAASGLIVSSNYMTWVRQAPGKGLEWVSVLYAGGSSFYADSVKGRFTISRDNSKNTLFLQMNSLRAEDTAVYYCARDLVAYGMDVWGQGTTVSVSSASTKGPSVFPLAPSSKSTSGGTAALGCLVKDYFPEPVTVSWNSGALTSGVHTFPAVLQSSGLYSLSSVVTVPSSSLGTQTYICNVNHKPSNTKVDKKVEPKSCDKTHTCPPCPAPELLGGPSVFLFPPKPKDTLMISRTPEVTCVVVDVSHEDPEVKFNWYVDGVEVHNAKTKPREEQYNSTYRVVSVLTVLHQDWLNGKEYKCKVSNKALPAPIEKTISKAKGQPREPQVYTLPPSRDELTKNQVSLTCLVKGFYPSDIAVEWESNGQPENNYKTTPPVLDSDGSFFLYSKLTVDKSRWQQGNVFSCSVMHEALHNHYTQKSLSLSPGK

SEQ ID NO: 138 - protein, 214 aa, Artificial Sequence
  Complete light chain of antibody R568-1B3 with IGKC*01
DIQLTQSPSFLSASVGGRVTITCRASQGISSSLAWYQQKPGKAPKLLIYGASTLRTGVPSRFSGSGSGTEFTLTISSLQPEDFATYYCQQLNSDLYTFGQGTKLEIKRTVAAPSVFIFPPSDEQLKSGTASVVCLLNNFYPREAKVQWKVDNALQSGNSQESVTEQDSKDSTYSLSSTLTLSKADYEKHKVYACEVTHQGLSSPVTKSFNRGEC

SEQ ID NO: 139 - protein, 447 aa, Artificial Sequence
  Complete heavy chain of antibody R568-2E1 with IGHG1*01
EVQLVESGGGLIQPGGSLRLSCAASGLTVSSNYMNWVRQAPGKGLEWVSVIYSGGTTYYADSVKGRFTISRDNSKNTLYLQMNNLRDEDTAMYYCARDLIVYGMDVWGQGTPVTVSSASTKGPSVFPLAPSSKSTSGGTAALGCLVKDYFPEPVTVSWNSGALTSGVHTFPAVLQSSGLYSLSSVVTVPSSSLGTQTYICNVNHKPSNTKVDKKVEPKSCDKTHTCPPCPAPELLGGPSVFLFPPKPKDTLMISRTPEVTCVVVDVSHEDPEVKFNWYVDGVEVHNAKTKPREEQYNSTYRVVSVLTVLHQDWLNGKEYKCKVSNKALPAPIEKTISKAKGQPREPQVYTLPPSRDELTKNQVSLTCLVKGFYPSDIAVEWESNGQPENNYKTTPPVLDSDGSFFLYSKLTVDKSRWQQGNVFSCSVMHEALHNHYTQKSLSLSPGK

SEQ ID NO: 140 - protein, 214 aa, Artificial Sequence
  Complete light chain of antibody R568-2E1 with IGKC*01
DIQLTQSPSFLSASVGDRVTITCRASQGISNYLAWYQQKPGKAPKLLIYGASTLQSGVPSRFSGSGSGTEFTLTISSLQPEDFATYYCQQLNSDFFTFGPGTKVDIKRTVAAPSVFIFPPSDEQLKSGTASVVCLLNNFYPREAKVQWKVDNALQSGNSQESVTEQDSKDSTYSLSSTLTLSKADYEKHKVYACEVTHQGLSSPVTKSFNRGEC

SEQ ID NO: 141 - protein, 448 aa, Artificial Sequence
  Complete heavy chain of antibody R568-1G9 with IGHG1*01
EVQLVESGGGLVQPGGSLRLSCAASGITVSSNYMSWVRQAPGKGLEWVSVIYSGGSTFYTDSVKGRFTISRDNSKNTLYLQMNSLRAEDTAVYYCARDLVVLYGMDVWGQGTTVTVSSASTKGPSVFPLAPSSKSTSGGTAALGCLVKDYFPEPVTVSWNSGALTSGVHTFPAVLQSSGLYSLSSVVTVPSSSLGTQTYICNVNHKPSNTKVDKKVEPKSCDKTHTCPPCPAPELLGGPSVFLFPPKPKDTLMISRTPEVTCVVVDVSHEDPEVKFNWYVDGVEVHNAKTKPREEQYNSTYRVVSVLTVLHQDWLNGKEYKCKVSNKALPAPIEKTISKAKGQPREPQVYTLPPSRDELTKNQVSLTCLVKGFYPSDIAVEWESNGQPENNYKTTPPVLDSDGSFFLYSKLTVDKSRWQQGNVFSCSVMHEALHNHYTQKSLSLSPGK

SEQ ID NO: 142 - protein, 216 aa, Artificial Sequence
  Complete light chain of antibody R568-1G9 with IGLC2*01
QSVLTQPPSVSGAPGQRVTISCTGNSSNIGAGYDVHWYQQLPGTAPKLLIYGNSNRPSGVPDRFSGSKSGTSASLAITGLQAEDEADYYCQSYDSSLSALFGTGTKVTVLGQPKAAPSVTLFPPSSEELQANKATLVCLISDFYPGAVTVAWKADSSPVKAGVETTTPSKQSNNKYAASSYLSLTPEQWKSHRSYSCQVTHEGSTVEKTVAPTECS

SEQ ID NO: 143 - protein, 451 aa, Artificial Sequence
  Complete heavy chain of antibody R121-1F1 with IGHG1*01
QVQLVESGGGVVQPERSLRLSCAASGFTFSRDGMHWVRRAPGKGLEWVAVISYDGSNKVYAESVKGRFTVSRDSSKNTVYLQMNSLRAEDTAVYYCAKDGPQAFGTYFDYWGQGTLVIVSSASTKGPSVFPLAPSSKSTSGGTAALGCLVKDYFPEPVTVSWNSGALTSGVHTFPAVLQSSGLYSLSSVVTVPSSSLGTQTYICNVNHKPSNTKVDKKVEPKSCDKTHTCPPCPAPELLGGPSVFLFPPKPKDTLMISRTPEVTCVVVDVSHEDPEVKFNWYVDGVEVHNAKTKPREEQYNSTYRVVSVLTVLHQDWLNGKEYKCKVSNKALPAPIEKTISKAKGQPREPQVYTLPPSRDELTKNQVSLTCLVKGFYPSDIAVEWESNGQPENNYKTTPPVLDSDGSFFLYSKLTVDKSRWQQGNVFSCSVMHEALHNHYTQKSLSLSPGK

SEQ ID NO: 144 - protein, 217 aa, Artificial Sequence
  Complete light chain of antibody R121-1F1 with  IGLC2*01
QSALTQPPSVSGAPGQRVTISCTGSSSNIGSGYVVHWYQHLPNTAPKLLIFGNNNRPSGVPDRFSGSKSGTSASLAITGLQAEDEADYYCQSYDSRLSGVVFGGGTKLTVLGQPKAAPSVTLFPPSSEELQANKATLVCLISDFYPGAVTVAWKADSSPVKAGVETTTPSKQSNNKYAASSYLSLTPEQWKSHRSYSCQVTHEGSTVEKTVAPTECS

SEQ ID NO: 145 - protein, 453 aa, Artificial Sequence
  Complete heavy chain of antibody R259-1B9 with IGHG1*01
QMHLVQSGPEVKKPGTSVKVSCKASGFTFSSSAVQWVRQARGQHLEWIGWIVVGSGNTNYGQKFQERVTITRDLSTSTVYMELISLRSEDTAVYFCAAPYCTGGSCFDAFDIWGQGTMVTVSSASTKGPSVFPLAPSSKSTSGGTAALGCLVKDYFPEPVTVSWNSGALTSGVHTFPAVLQSSGLYSLSSVVTVPSSSLGTQTYICNVNHKPSNTKVDKKVEPKSCDKTHTCPPCPAPELLGGPSVFLFPPKPKDTLMISRTPEVTCVVVDVSHEDPEVKFNWYVDGVEVHNAKTKPREEQYNSTYRVVSVLTVLHQDWLNGKEYKCKVSNKALPAPIEKTISKAKGQPREPQVYTLPPSRDELTKNQVSLTCLVKGFYPSDIAVEWESNGQPENNYKTTPPVLDSDGSFFLYSKLTVDKSRWQQGNVFSCSVMHEALHNHYTQKSLSLSPGK

SEQ ID NO: 146 - protein, 215 aa, Artificial Sequence
  Complete light chain of antibody R259-1B9 with IGKC*01
ETVLTQSPGTLSLSPGERATLSCRASQSVRSSYLAWYQQKPGQAPRLVIYGPSTRATGIPDRFSGSGSGTDFTLTISRLEPEDFAVYYCQQYGSSPWTFGQGTKVEIKRTVAAPSVFIFPPSDEQLKSGTASVVCLLNNFYPREAKVQWKVDNALQSGNSQESVTEQDSKDSTYSLSSTLTLSKADYEKHKVYACEVTHQGLSSPVTKSFNRGEC

SEQ ID NO: 147 - protein, 459 aa, Artificial Sequence
  Complete heavy chain of antibody R121-3G2 with IGHG1*01
QLQLQESGPGLVKPSETLSLTCTVSGGSIASTYYYWGWIRQSPGKGLEWIANIHYNGSTYNKPSLKNRVTLSVDTSKNQFSLKLSSVTAADTAVYYCARYGPYYYDRSGSLLSDPFDNWGQGTLVTVSSASTKGPSVFPLAPSSKSTSGGTAALGCLVKDYFPEPVTVSWNSGALTSGVHTFPAVLQSSGLYSLSSVVTVPSSSLGTQTYICNVNHKPSNTKVDKKVEPKSCDKTHTCPPCPAPELLGGPSVFLFPPKPKDTLMISRTPEVTCVVVDVSHEDPEVKFNWYVDGVEVHNAKTKPREEQYNSTYRVVSVLTVLHQDWLNGKEYKCKVSNKALPAPIEKTISKAKGQPREPQVYTLPPSRDELTKNQVSLTCLVKGFYPSDIAVEWESNGQPENNYKTTPPVLDSDGSFFLYSKLTVDKSRWQQGNVFSCSVMHEALHNHYTQKSLSLSPGK

SEQ ID NO: 148 - protein, 215 aa, Artificial Sequence
  Complete light chain of antibody R121-3G2 with IGKC*01
EVVLTQSPGTLSLSPGERATLSCRASQGLSSSSLAWYQQRPGQAPRLLIYGASNRATGISDRFSGSGSGTDFTLSVSRLEPEDFAVYYCQQYSNSPLTFGQGTKVEIKRTVAAPSVFIFPPSDEQLKSGTASVVCLLNNFYPREAKVQWKVDNALQSGNSQESVTEQDSKDSTYSLSSTLTLSKADYEKHKVYACEVTHQGLSSPVTKSFNRGEC

SEQ ID NO: 149 - protein, 461 aa, Artificial Sequence
  Complete heavy chain of antibody R40-1E1 with IGHG1*01
QVQLVESGGGVVQPGRSLRLSCAASGFTFSRYGMNWVRQAPGKGLEWVAVIWYDGNNKYYADSVKGRFTISRDNSKTTLYLQMKSLRAEDTAVYYCARALQYYDILTGDYSVVRSDAFDIWGQGTMVTVSSASTKGPSVFPLAPSSKSTSGGTAALGCLVKDYFPEPVTVSWNSGALTSGVHTFPAVLQSSGLYSLSSVVTVPSSSLGTQTYICNVNHKPSNTKVDKKVEPKSCDKTHTCPPCPAPELLGGPSVFLFPPKPKDTLMISRTPEVTCVVVDVSHEDPEVKFNWYVDGVEVHNAKTKPREEQYNSTYRVVSVLTVLHQDWLNGKEYKCKVSNKALPAPIEKTISKAKGQPREPQVYTLPPSRDELTKNQVSLTCLVKGFYPSDIAVEWESNGQPENNYKTTPPVLDSDGSFFLYSKLTVDKSRWQQGNVFSCSVMHEALHNHYTQKSLSLSPGK

SEQ ID NO: 150 - protein, 215 aa, Artificial Sequence
  Complete light chain of antibody R40-1E1 with IGKC*01
EIVLTQSPGTLSLSPGERATLSCRASQSVSGTYLAWYQQKPGQAPRLLIYGASSRASGIPDRFSGSGSGTDFTLTISRLEPEDFAVYYCQQYGSSPLTFGGGTKVEIKRTVAAPSVFIFPPSDEQLKSGTASVVCLLNNFYPREAKVQWKVDNALQSGNSQESVTEQDSKDSTYSLSSTLTLSKADYEKHKVYACEVTHQGLSSPVTKSFNRGEC

SEQ ID NO: 151 - protein, 1208 aa, Artificial Sequence
  Ectodomain of the spike (S) homotrimer of SARS-CoV-2 in the Hexapro prefusion-stabilized-variant of the virus isolate Wuhan-Hu-1 as described in Hsieh et al., Science (2020) doi: 10.1126/science.abd0826
MFVFLVLLPLVSSQCVNLTTRTQLPPAYTNSFTRGVYYPDKVFRSSVLHSTQDLFLPFFSNVTWFHAIHVSGTNGTKRFDNPVLPFNDGVYFASTEKSNIIRGWIFGTTLDSKTQSLLIVNNATNVVIKVCEFQFCNDPFLGVYYHKNNKSWMESEFRVYSSANNCTFEYVSQPFLMDLEGKQGNFKNLREFVFKNIDGYFKIYSKHTPINLVRDLPQGFSALEPLVDLPIGINITRFQTLLALHRSYLTPGDSSSGWTAGAAAYYVGYLQPRTFLLKYNENGTITDAVDCALDPLSETKCTLKSFTVEKGIYQTSNFRVQPTESIVRFPNITNLCPFGEVFNATRFASVYAWNRKRISNCVADYSVLYNSASFSTFKCYGVSPTKLNDLCFTNVYADSFVIRGDEVRQIAPGQTGKIADYNYKLPDDFTGCVIAWNSNNLDSKVGGNYNYLYRLFRKSNLKPFERDISTEIYQAGSTPCNGVEGFNCYFPLQSYGFQPTNGVGYQPYRVVVLSFELLHAPATVCGPKKSTNLVKNKCVNFNFNGLTGTGVLTESNKKFLPFQQFGRDIADTTDAVRDPQTLEILDITPCSFGGVSVITPGTNTSNQVAVLYQDVNCTEVPVAIHADQLTPTWRVYSTGSNVFQTRAGCLIGAEHVNNSYECDIPIGAGICASYQTQTNSPGSASSVASQSIIAYTMSLGAENSVAYSNNSIAIPTNFTISVTTEILPVSMTKTSVDCTMYICGDSTECSNLLLQYGSFCTQLNRALTGIAVEQDKNTQEVFAQVKQIYKTPPIKDFGGFNFSQILPDPSKPSKRSPIEDLLFNKVTLADAGFIKQYGDCLGDIAARDLICAQKFNGLTVLPPLLTDEMIAQYTSALLAGTITSGWTFGAGPALQIPFPMQMAYRFNGIGVTQNVLYENQKLIANQFNSAIGKIQDSLSSTPSALGKLQDVVNQNAQALNTLVKQLSSNFGAISSVLNDILSRLDPPEAEVQIDRLITGRLQSLQTYVTQQLIRAAEIRASANLAATKMSECVLGQSKRVDFCGKGYHLMSFPQSAPHGVVFLHVTYVPAQEKNFTTAPAICHDGKAHFPREGVFVSNGTHWFVTQRNFYEPQIITTDNTFVSGNCDVVIGIVNNTVYDPLQPELDSFKEELDKYFKNHTSPDVDLGDISGINASVVNIQKEIDRLNEVAKNLNESLIDLQELGKYEQ

SEQ ID NO: 152 - protein, 223 aa, Artificial Sequence
  Receptor-binding domain (RBD) of the spike (S) protein of SARS-CoV-2 of the virus isolate Wuhan-Hu-1 as described in Wrapp et al., Science (2022) doi: 10.1126/science.abb2507
RVQPTESIVRFPNITNLCPFGEVFNATRFASVYAWNRKRISNCVADYSVLYNSASFSTFKCYGVSPTKLNDLCFTNVYADSFVIRGDEVRQIAPGQTGKIADYNYKLPDDFTGCVIAWNSNNLDSKVGGNYNYLYRLFRKSNLKPFERDISTEIYQAGSTPCNGVEGFNCYFPLQSYGFQPTNGVGYQPYRVVVLSFELLHAPATVCGPKKSTNLVKNKCVNF